European Patent Application EP 4 682 146 A1, published January 21, 2026. Title: A Composition for Preventing or Treating Neurodegenerative Diseases Comprising Novel Pyridoindole Derivatives As Active Ingredients. Applicant: Korea Institute of Science and Technology. Application KR. The sequence listing filed with the application follows.

SEQUENCE LISTING (14 sequences)

SEQ ID NO: 1 - DNA, 43 bp, synthetic construct
  source 1..43: mol_type = other DNA
atgaggtacctcttctagagccaccatggctgagccccgccag

SEQ ID NO: 2 - DNA, 61 bp, synthetic construct
  source 1..61: mol_type = other DNA
ttatgggccctgcggccgcacttcagaattcacctgcggatcccaaaccctgcttggccag

SEQ ID NO: 3 - DNA, 67 bp, synthetic construct
  source 1..67: mol_type = other DNA
atgaggtacctcttctagagacatcctcgagaatgtaggatccgccaccatggctgagccccgccag

SEQ ID NO: 4 - DNA, 43 bp, synthetic construct
  source 1..43: mol_type = other DNA
ttatgggccctgcggccgcacttcacaaaccctgcttggccag

SEQ ID NO: 5 - DNA, 51 bp, synthetic construct
  source 1..51: mol_type = other DNA
aataggatcctcaggcagctctagagccaccatggtgagcaagggcgagga

SEQ ID NO: 6 - DNA, 46 bp, synthetic construct
  source 1..46: mol_type = other DNA
ataaggatccgcttccgctgaattccttgtacagctcgtccatgcc

SEQ ID NO: 7 - DNA, 35 bp, synthetic construct
  source 1..35: mol_type = other DNA
aattctagagccaccatggtgaccggctatcgcct

SEQ ID NO: 8 - DNA, 35 bp, synthetic construct
  source 1..35: mol_type = other DNA
attattgaattcctacaaaccctgcttggccaggg

SEQ ID NO: 9 - DNA, 48 bp, synthetic construct
  source 1..48: mol_type = other DNA
aatggtacctccgcactcgaggccaccatggctgagccccgccaggag

SEQ ID NO: 10 - DNA, 42 bp, synthetic construct
  source 1..42: mol_type = other DNA
gccgattccggcctcctcggcttccgctgttggagtgctctt

SEQ ID NO: 11 - DNA, 42 bp, synthetic construct
  source 1..42: mol_type = other DNA
gccgaggaggccggaatcggcgacacccccagcctggaagac

SEQ ID NO: 12 - DNA, 43 bp, synthetic construct
  source 1..43: mol_type = other DNA
aatagaattcggcagcggatcccaaaccctgcttggccaggga

SEQ ID NO: 13 - DNA, 73 bp, synthetic construct
  source 1..73: mol_type = other DNA
aagagatctcagtatttacaaacaaccatgaatgtaagtatattccgtcgacgtcgagctcggtacccgggtc

SEQ ID NO: 14 - DNA, 71 bp, synthetic construct
  source 1..71: mol_type = other DNA
aatctagagctttagaattcgctttaggatccgctaagcttgctgctctcgaggctccctatagtgagtcg